European Patent Specification EP 3 998 285 B1, published January 22, 2025. Title: Binding molecules to CD38 and PD-L1. Applicant: Biomunex pharmaceuticals. The sequence listing filed with the application follows.

SEQUENCE LISTING (32 sequences)

SEQ ID NO: 1 - protein, 709 aa, Artificial Sequence
  BiXAb 4218 heavy chain
EVQLLESGGGLVQPGGSLRLSCAVSGFTFNSFAMSWVRQAPGKGLEWVSAISGSGGGTYYADSVKGRFTISRDNSKNTLYLQMNSLRAEDTAVYFCAKDKILWFGEPVFDYWGQGTLVTVSSASTKGPSVFPLAPSSKSTSGGTAALGCLVKDYFPEPVTVSWNSGALTSGVHTFPAVLQSSGLYSLSSVVKVPSSSLGTQTYICNVNHKPSNTKVDKRVEPKSCDKTHTCPPCPAPELLGGPSTPPTPSPSGGENLYFQGEVQLVESGGGLVQPGGSLRLSCAASGFTFSDSWIHWVRQAPGKGLEWVAWISPYGGSTYYADSVKGRFTISADTSKNTAYLQMNSLRAEDTAVYYCARRHWPGGFDYWGQGTLVTVSSASTKGPSVFPLAPSSKSTSGGTAALGCLVKDYFPEPVTVSWNSGALTSGVHTFPAVLQSSGLYSLSSVVEVPSSSLGTQTYICNVNHKPSNTKVDKKVEPKSCDKTHTCPPCPAPELLGGPSVFLFPPKPKDTLMISRTPEVTCVVVDVSHEDPEVKFNWYVDGVEVHNAKTKPREEQYNSTYRVVSVLTVLHQDWLNGKEYKCKVSNKALPAPIEKTISKAKGQPREPQVYTLPPSREEMTKNQVSLTCLVKGFYPSDIAVEWESNGQPENNYKTTPPVLDSDGSFFLYSKLTVDKSRWQQGNVFSCSVMHEALHNHYTQKSLSLSPGK

SEQ ID NO: 2 - protein, 214 aa, Artificial Sequence
  LC1
EIVLTQSPATLSLSPGERATLSCRASQSVSSYLAWYQQKPGQAPRLLIYDASNRATGIPARFSGSGSGTDFTLTISSLEPEDFAVYYCQQRSNWPPTFGQGTKVEIKRTVAAPAVFIFPPSDEQLKSGTASVVCLLENFYPREAKVQWKVDNALQSGNSQESVTEQDSKDSTYSLSSTLTLSKADYEKHKVYACEVTHQGLSSPVTKSFNRGEC

SEQ ID NO: 3 - protein, 214 aa, Artificial Sequence
  LC2
DIQMTQSPSSLSASVGDRVTITCRASQDVSTAVAWYQQKPGKAPKLLIYSASFLYSGVPSRFSGSGSGTDFTLTISSLQPEDFATYYCQQYLYHPATFGQGTKVEIKRTVAAPAVFIFPPSDEQLKSGTASVVCLLKNFYPREAKVQWKVDNALQSGNSQESVTEQDSKDSTYSLSSTLTLSKADYEKHKVYACEVTHQGLSSPVTKSFNRGEC

SEQ ID NO: 4 - protein, 709 aa, Artificial Sequence
  BiXAb 4219 Heavy chain
EVQLVESGGGLVQPGGSLRLSCAASGFTFSDSWIHWVRQAPGKGLEWVAWISPYGGSTYYADSVKGRFTISADTSKNTAYLQMNSLRAEDTAVYYCARRHWPGGFDYWGQGTLVTVSSASTKGPSVFPLAPSSKSTSGGTAALGCLVKDYFPEPVTVSWNSGALTSGVHTFPAVLQSSGLYSLSSVVEVPSSSLGTQTYICNVNHKPSNTKVDKRVEPKSCDKTHTCPPCPAPELLGGPSTPPTPSPSGGENLYFQGEVQLLESGGGLVQPGGSLRLSCAVSGFTFNSFAMSWVRQAPGKGLEWVSAISGSGGGTYYADSVKGRFTISRDNSKNTLYLQMNSLRAEDTAVYFCAKDKILWFGEPVFDYWGQGTLVTVSSASTKGPSVFPLAPSSKSTSGGTAALGCLVKDYFPEPVTVSWNSGALTSGVHTFPAVLQSSGLYSLSSVVKVPSSSLGTQTYICNVNHKPSNTKVDKKVEPKSCDKTHTCPPCPAPELLGGPSVFLFPPKPKDTLMISRTPEVTCVVVDVSHEDPEVKFNWYVDGVEVHNAKTKPREEQYNSTYRVVSVLTVLHQDWLNGKEYKCKVSNKALPAPIEKTISKAKGQPREPQVYTLPPSREEMTKNQVSLTCLVKGFYPSDIAVEWESNGQPENNYKTTPPVLDSDGSFFLYSKLTVDKSRWQQGNVFSCSVMHEALHNHYTQKSLSLSPGK

SEQ ID NO: 5 - protein, 214 aa, Artificial Sequence; identical to SEQ ID NO: 3
  LC1

SEQ ID NO: 6 - protein, 214 aa, Artificial Sequence; identical to SEQ ID NO: 2
  LC2

SEQ ID NO: 7 - protein, 710 aa, Artificial Sequence
  BiXAb 5104 Heavy chain
QVQLVQSGAEVAKPGTSVKLSCKASGYTFTDYWMQWVKQRPGQGLEWIGTIYGPDGDTGYAQKFQGKATLTADKSSKTVYMHLSSLASEDSAVYYCARGDYYGSNSLDYWGQGTSVTVSSASTKGPSVFPLAPSSKSTSGGTAALGCLVKDYFPEPVTVSWNSGALTSGVHTFPAVLQSSGLYSLSSVVKVPSSSLGTQTYICNVNHKPSNTKVDKRVEPKSCDKTHTCPPCPAPELLGGPSTPPTPSPSGGENLYFQGEVQLVESGGGLVQPGGSLRLSCAASGFTFSRYWMSWVRQAPGKGLEWVANIKQDGSEKYYVDSVKGRFTISRDNAKNSLYLQMNSLRAEDTAVYYCAREGGWFGELAFDYWGQGTLVTVSSASTKGPSVFPLAPSSKSTSGGTAALGCLVKDYFPEPVTVSWNSGALTSGVHTFPAVLQSSGLYSLSSVVEVPSSSLGTQTYICNVNHKPSNTKVDKKVEPKSCDKTHTCPPCPAPELLGGPSVFLFPPKPKDTLMISRTPEVTCVVVDVSHEDPEVKFNWYVDGVEVHNAKTKPREEQYNSTYRVVSVLTVLHQDWLNGKEYKCKVSNKALPAPIEKTISKAKGQPREPQVYTLPPSREEMTKNQVSLTCLVKGFYPSDIAVEWESNGQPENNYKTTPPVLDSDGSFFLYSKLTVDKSRWQQGNVFSCSVMHEALHNHYTQKSLSLSPGK

SEQ ID NO: 8 - protein, 214 aa, Artificial Sequence
  LC1
DIVMTQSHLSMSTSLGDPVSITCKASQDVSTVVAWYQQKPGQSPRRLIYSASYRYIGVPDRFTGSGAGTDFTFTISSVQAEDLAVYYCQQHYSPPYTFGGGTKLEIKRTVAAPAVFIFPPSDEQLKSGTASVVCLLENFYPREAKVQWKVDNALQSGNSQESVTEQDSKDSTYSLSSTLTLSKADYEKHKVYACEVTHQGLSSPVTKSFNRGEC

SEQ ID NO: 9 - protein, 215 aa, Artificial Sequence
  LC2
EIVLTQSPGTLSLSPGERATLSCRASQRVSSSYLAWYQQKPGQAPRLLIYDASSRATGIPDRFSGSGSGTDFTLTISRLEPEDFAVYYCQQYGSLPWTFGQGTKVEIKRTVAAPAVFIFPPSDEQLKSGTASVVCLLKNFYPREAKVQWKVDNALQSGNSQESVTEQDSKDSTYSLSSTLTLSKADYEKHKVYACEVTHQGLSSPVTKSFNRGEC

SEQ ID NO: 10 - protein, 702 aa, Artificial Sequence
  BiXAB BMX101-AP-ML1-CC1
EVQLLESGGGLVQPGGSLRLSCAVSGFTFNSFAMSWVRQAPGKGLEWVSAISGSGGGTYYADSVKGRFTISRDNSKNTLYLQMNSLRAEDTAVYFCAKDKILWFGEPVFDYWGQGTLVTVSSASTKGPSVFPQAPSSKSTSGGTAALGCLVKDYFPEPVTVSWNSGALTSGVHTFPAVLQSSGLYSLVSVVTVPSSSLGTQTYICNVNHKPSNTKVDKRVEPKSCDKTHTSPPAPAPELLGGPAAPPAPAPAGGEVQLVESGGGLVQPGGSLRLSCAASGFTFSDSWIHWVRQAPGKGLEWVAWISPYGGSTYYADSVKGRFTISADTSKNTAYLQMNSLRAEDTAVYYCARRHWPGGFDYWGQGTLVTVSSASTKGPSVFPLAPSSKSTSGGTAALGCLVKDYFPEPVTVSWNSGALTSGVHTFPAVLQSSGLYSLSSVVDVPSSSLGTQTYICNVNHKPSNTKVDKRVEPKSCDKTHTCPPCPAPELLGGPSVFLFPPKPKDTLMISRTPEVTCVVVDVSHEDPEVKFNWYVDGVEVHNAKTKPREEQYNSTYRVVSVLTVLHQDWLNGKEYKCKVSNKALPAPIEKTISKAKGQPREPQVYTLPPSREEMTKNQVSLTCLVKGFYPSDIAVEWESNGQPENNYKTTPPVLDSDGSFFLYSKLTVDKSRWQQGNVFSCSVMHEALHNHYTQKSLSLSPGK

SEQ ID NO: 11 - protein, 214 aa, Artificial Sequence
  Daratumumab LC
EIVLTQSPATLSLSPGERATLSCRASQSVSSYLAWYQQKPGQAPRLLIYDASNRATGIPARFSGSGSGTDFTLTISSLEPEDFAVYYCQQRSNWPPTFGQGTKVEIKRTVAAPSVFIFPPSDEQLKSGTASVTCLLNNFYPREAKVQWKVDNALQSGNSQESVTEQDSKDSTYSLVSTLTLSKADYEKHKVYACEVTHQGLSSPVTKSFNRGEC

SEQ ID NO: 12 - protein, 214 aa, Artificial Sequence; identical to SEQ ID NO: 3
  Atezolizumab-LC

SEQ ID NO: 13 - protein, 34 aa, Artificial Sequence
  Linker 1
  misc_feature (4)..(4): Xaa can be any naturally occurring amino acid
  misc_feature (8)..(8): Xaa can be any naturally occurring amino acid
  misc_feature (10)..(11): Xaa can be any naturally occurring amino acid
  misc_feature (14)..(14): Xaa can be any naturally occurring amino acid
  misc_feature (24)..(25): Xaa can be any naturally occurring amino acid
  misc_feature (28)..(28): Xaa can be any naturally occurring amino acid
  misc_feature (30)..(30): Xaa can be any naturally occurring amino acid
  misc_feature (32)..(32): Xaa can be any naturally occurring amino acid
EPKXCDKXHXXPPXPAPELLGGPXXPPXPXPXGG

SEQ ID NO: 14 - protein, 34 aa, Artificial Sequence
  Linker 2
EPKSCDKTHTSPPAPAPELLGGPGGPPGPGPGGG

SEQ ID NO: 15 - protein, 34 aa, Artificial Sequence
  Linker 2
EPKSCDKTHTSPPAPAPELLGGPAAPPAPAPAGG

SEQ ID NO: 16 - protein, 34 aa, Artificial Sequence
  Linker 3
EPKSCDKTHTSPPAPAPELLGGPAAPPGPAPGGG

SEQ ID NO: 17 - protein, 34 aa, Artificial Sequence
  Linker 4
EPKSCDKTHTCPPCPAPELLGGPSTPPTPSPSGG

SEQ ID NO: 18 - protein, 34 aa, Artificial Sequence
  Linker 6
EPKSCDKTHTSPPSPAPELLGGPSTPPTPSPSGG

SEQ ID NO: 19 - protein, 9 aa, Artificial Sequence
  Nter IgG1 CH2
APELLGGPS

SEQ ID NO: 20 - protein, 8 aa, Artificial Sequence
  Portion of human IgA1 hinge
TPPTPSPS

SEQ ID NO: 21 - protein, 19 aa, Artificial Sequence
  signal peptide
MNFGLRLIFLVLTLKGVQC

SEQ ID NO: 22 - protein, 122 aa, Homo sapiens [sequence omitted]

SEQ ID NO: 23 - protein, 98 aa, Artificial Sequence
  CH1 domain of daratumumab
ASTKGPSVFPQAPSSKSTSGGTAALGCLVKDYFPEPVTVSWNSGALTSGVHTFPAVLQSSGLYSLVSVVTVPSSSLGTQTYICNVNHKPSNTKVDKRV

SEQ ID NO: 24 - protein, 118 aa, Artificial Sequence [sequence omitted]

SEQ ID NO: 25 - protein, 98 aa, Artificial Sequence
  CH1 domain of atezolizumab
ASTKGPSVFPLAPSSKSTSGGTAALGCLVKDYFPEPVTVSWNSGALTSGVHTFPAVLQSSGLYSLSSVVDVPSSSLGTQTYICNVNHKPSNTKVDKRV

SEQ ID NO: 26 - protein, 15 aa, Homo sapiens
EPKSCDKTHTCPPCP

SEQ ID NO: 27 - protein, 110 aa, Homo sapiens
APELLGGPSVFLFPPKPKDTLMISRTPEVTCVVVDVSHEDPEVKFNWYVDGVEVHNAKTKPREEQYNSTYRVVSVLTVLHQDWLNGKEYKCKVSNKALPAPIEKTISKAK

SEQ ID NO: 28 - protein, 107 aa, Homo sapiens
GQPREPQVYTLPPSREEMTKNQVSLTCLVKGFYPSDIAVEWESNGQPENNYKTTPPVLDSDGSFFLYSKLTVDKSRWQQGNVFSCSVMHEALHNHYTQKSLSLSPGK

SEQ ID NO: 29 - protein, 107 aa, Homo sapiens [sequence omitted]

SEQ ID NO: 30 - protein, 107 aa, Artificial Sequence
  CKappa domain of daratumumab
RTVAAPSVFIFPPSDEQLKSGTASVTCLLNNFYPREAKVQWKVDNALQSGNSQESVTEQDSKDSTYSLVSTLTLSKADYEKHKVYACEVTHQGLSSPVTKSFNRGEC

SEQ ID NO: 31 - protein, 107 aa, Artificial Sequence [sequence omitted]

SEQ ID NO: 32 - protein, 107 aa, Artificial Sequence
  CKappa domain of atezolizumab
RTVAAPAVFIFPPSDEQLKSGTASVVCLLKNFYPREAKVQWKVDNALQSGNSQESVTEQDSKDSTYSLSSTLTLSKADYEKHKVYACEVTHQGLSSPVTKSFNRGEC